European Patent Application EP 4 349 856 A1, published April 10, 2024. Title: DEVELOPMENT AND USE OF NOVEL INTERLEUKIN 15 MUTANT POLYPEPTIDE. Applicant: Suzhou Forlong Biotechnology Co., Ltd. Application EP 22810503.7. The sequence listing filed with the application follows.

SEQUENCE LISTING (17 sequences)

SEQ ID NO: 1 - protein, 114 aa, Artificial Sequence(2 Ambystoma laterale x Ambystoma jeffersonianum)
NWVXVIXXLKKIEDLIQSMHIDATLYTESDVHPSCKVTAMKCFLLELQVISLESGDASIHXTVXNLIXLANXSLSSNGNVTESGCKECEELEEKNIKEFLQSFVHIVXXFXNTS

SEQ ID NO: 2 - protein, 114 aa, Artificial Sequence(2 Ambystoma laterale x Ambystoma jeffersonianum)
NWVAVISDLKKIEDLIQSMHIDATLYTESDVHPSCKVTAMKCFLLELQVISLESGDASIHDTVENLIILANNSLSSNGNVTESGCKECEELEEKNIKEFLQSFVHIVQMFINTS

SEQ ID NO: 3 - protein, 114 aa, Artificial Sequence(2 Ambystoma laterale x Ambystoma jeffersonianum)
NWVNVIDDLKKIEDLIQSMHIDATLYTESDVHPSCKVTAMKCFLLELQVISLESGDASIHDTVENLIILANNSLSSNGNVTESGCKECEELEEKNIKEFLQSFVHIVQMFINTS

SEQ ID NO: 4 - protein, 114 aa, Artificial Sequence(2 Ambystoma laterale x Ambystoma jeffersonianum)
NWVNVIYDLKKIEDLIQSMHIDATLYTESDVHPSCKVTAMKCFLLELQVISLESGDASIHDTVENLIILANNSLSSNGNVTESGCKECEELEEKNIKEFLQSFVHIVQMFINTS

SEQ ID NO: 5 - protein, 114 aa, Artificial Sequence(2 Ambystoma laterale x Ambystoma jeffersonianum)
NWVNVISFLKKIEDLIQSMHIDATLYTESDVHPSCKVTAMKCFLLELQVISLESGDASIHDTVENLIILANNSLSSNGNVTESGCKECEELEEKNIKEFLQSFVHIVQMFINTS

SEQ ID NO: 6 - protein, 114 aa, Artificial Sequence(2 Ambystoma laterale x Ambystoma jeffersonianum)
NWVNVISDLKKIEDLIQSMHIDATLYTESDVHPSCKVTAMKCFLLELQVISLESGDASIHGTVENLIILANNSLSSNGNVTESGCKECEELEEKNIKEFLQSFVHIVQMFINTS

SEQ ID NO: 7 - protein, 114 aa, Artificial Sequence(2 Ambystoma laterale x Ambystoma jeffersonianum)
NWVNVISDLKKIEDLIQSMHIDATLYTESDVHPSCKVTAMKCFLLELQVISLESGDASIHNTVENLIILANNSLSSNGNVTESGCKECEELEEKNIKEFLQSFVHIVQMFINTS

SEQ ID NO: 8 - protein, 114 aa, Artificial Sequence(2 Ambystoma laterale x Ambystoma jeffersonianum)
NWVNVISDLKKIEDLIQSMHIDATLYTESDVHPSCKVTAMKCFLLELQVISLESGDASIHDTVYNLIILANNSLSSNGNVTESGCKECEELEEKNIKEFLQSFVHIVQMFINTS

SEQ ID NO: 9 - protein, 114 aa, Artificial Sequence(2 Ambystoma laterale x Ambystoma jeffersonianum)
NWVNVISDLKKIEDLIQSMHIDATLYTESDVHPSCKVTAMKCFLLELQVISLESGDASIHDTVENLIQLANNSLSSNGNVTESGCKECEELEEKNIKEFLQSFVHIVQMFINTS

SEQ ID NO: 10 - protein, 114 aa, Artificial Sequence(2 Ambystoma laterale x Ambystoma jeffersonianum)
NWVNVISDLKKIEDLIQSMHIDATLYTESDVHPSCKVTAMKCFLLELQVISLESGDASIHDTVENLIKLANNSLSSNGNVTESGCKECEELEEKNIKEFLQSFVHIVQMFINTS

SEQ ID NO: 11 - protein, 114 aa, Artificial Sequence(2 Ambystoma laterale x Ambystoma jeffersonianum)
NWVNVISDLKKIEDLIQSMHIDATLYTESDVHPSCKVTAMKCFLLELQVISLESGDASIHDTVENLIILANYSLSSNGNVTESGCKECEELEEKNIKEFLQSFVHIVQMFINTS

SEQ ID NO: 12 - protein, 114 aa, Artificial Sequence(2 Ambystoma laterale x Ambystoma jeffersonianum)
NWVNVISDLKKIEDLIQSMHIDATLYTESDVHPSCKVTAMKCFLLELQVISLESGDASIHDTVENLIILANNSLSSNGNVTESGCKECEELEEKNIKEFLQSFVHIVSMFINTS

SEQ ID NO: 13 - protein, 114 aa, Artificial Sequence(2 Ambystoma laterale x Ambystoma jeffersonianum)
NWVNVISDLKKIEDLIQSMHIDATLYTESDVHPSCKVTAMKCFLLELQVISLESGDASIHDTVENLIILANNSLSSNGNVTESGCKECEELEEKNIKEFLQSFVHIVFMFINTS

SEQ ID NO: 14 - protein, 114 aa, Artificial Sequence(2 Ambystoma laterale x Ambystoma jeffersonianum)
NWVNVISDLKKIEDLIQSMHIDATLYTESDVHPSCKVTAMKCFLLELQVISLESGDASIHDTVENLIILANNSLSSNGNVTESGCKECEELEEKNIKEFLQSFVHIVAMFINTS

SEQ ID NO: 15 - protein, 114 aa, Artificial Sequence(2 Ambystoma laterale x Ambystoma jeffersonianum)
NWVNVISDLKKIEDLIQSMHIDATLYTESDVHPSCKVTAMKCFLLELQVISLESGDASIHDTVENLIILANNSLSSNGNVTESGCKECEELEEKNIKEFLQSFVHIVQHFINTS

SEQ ID NO: 16 - protein, 114 aa, Artificial Sequence(2 Ambystoma laterale x Ambystoma jeffersonianum)
NWVNVISDLKKIEDLIQSMHIDATLYTESDVHPSCKVTAMKCFLLELQVISLESGDASIHDTVENLIILANNSLSSNGNVTESGCKECEELEEKNIKEFLQSFVHIVQMFANTS

SEQ ID NO: 17 - protein, 114 aa, Artificial Sequence(2 Ambystoma laterale x Ambystoma jeffersonianum)
NWVNVISDLKKIEDLIQSMHIDATLYTESDVHPSCKVTAMKCFLLELQVISLESGDASIHDTVENLIILANNSLSSNGNVTESGCKECEELEEKNIKEFLQSFVHIVQMFHNTS